European Patent Application EP 4 631 528 A1, published October 15, 2025. Title: Nanoparticle Comprising Peptide-based Conjugate for Delivering Oligonucleotide into Target Cell and Pharmaceutical Composition Comprising Thereof. Applicant: NIBEC Co., Ltd. The sequence listing filed with the application follows.

SEQUENCE LISTING (21 sequences)

SEQ ID NO: 1 - protein, 16 aa, synthetic construct
LKKLLKLLKKLLKLAG

SEQ ID NO: 2 - protein, 16 aa, synthetic construct
IKKLIKIIKKLIKLAG

SEQ ID NO: 3 - protein, 16 aa, synthetic construct
LRRLLRLLRRLLRLAG

SEQ ID NO: 4 - protein, 16 aa, synthetic construct
  SITE 9: note = Ornithine
  SITE 13: note = 2,3-diaminopropionic acid
LKKLLKLLXKLLXLAG

SEQ ID NO: 5 - protein, 16 aa, synthetic construct
  SITE 9: note = Ornithine
  SITE 13: note = 2,3-diaminopropionic acid
LRRLLRLLXRLLXLAG

SEQ ID NO: 6 - protein, 16 aa, synthetic construct
  SITE 9: note = Ornithine
  SITE 13: note = 2,3-diaminopropionic acid
LRKIIRLIXKLLXLAG

SEQ ID NO: 7 - protein, 16 aa, synthetic construct
  SITE 9: note = Ornithine
LKKLLKLLXKLLKLAG

SEQ ID NO: 8 - protein, 16 aa, synthetic construct
WKKLLKLLKKLLKLAG

SEQ ID NO: 9 - protein, 16 aa, synthetic construct
WRRLLRLLRRLLRLAG

SEQ ID NO: 10 - protein, 16 aa, synthetic construct
WRKLLRLLKKLLKLAG

SEQ ID NO: 11 - protein, 16 aa, synthetic construct
  SITE 6: note = 2,4-diaminobutyric acid
LKKLLXLLKKLLKWAG

SEQ ID NO: 12 - protein, 16 aa, synthetic construct
  SITE 6: note = 2,4-diaminobutyric acid
LRRLLXLLRRLLRWAG

SEQ ID NO: 13 - protein, 16 aa, synthetic construct
  SITE 6: note = 2,4-diaminobutyric acid
LKRLIXIIKKLIKWAG

SEQ ID NO: 14 - protein, 16 aa, synthetic construct
  SITE 9: note = Ornithine
  SITE 13: note = 2,3-diaminopropionic acid
LKKLLKWLXKLLXLAG

SEQ ID NO: 15 - protein, 16 aa, synthetic construct
  SITE 9: note = Ornithine
  SITE 13: note = 2,4-diaminobutyric acid
LRRLLRWLXRLLXLAG

SEQ ID NO: 16 - protein, 8 aa, synthetic construct
MMIVRSQN

SEQ ID NO: 17 - protein, 7 aa, synthetic construct
CAIYPRH

SEQ ID NO: 18 - RNA, 1461 nt, synthetic construct
  source 1..1461: mol_type = other RNA
atggaagtccaattgttggaatctgggggtgggcttgtccaacctggtggttcactccgtctgagctgcgccgcttccggattcactttctccaccttttctatgaattgggttcgccaggccccaggcaagggacttgagtgggttagctatatcagcaggaccagtaaaaccatctactacgccgacagcgttaagggaaggttcactatatcccgggacaattctaagaatactttgtacttgcaaatgaactctttgcgggcagaagatactgctgtctactattgtgcacgaggtaggttttttgattattggggtcaggggaccctcgtaaccgtttccagtgggggcagcgagggtaagagctccggttcagggtcagaatctaaaagcactggtggctccgatatacaaatgacccagagtccaagctctctttcagccagcgtgggagacagggtgaccatcacctgtcgagcatctcaatccatttcatcatacctcaattggtatcaacagaagcctggggaagcaccaaagttgcttatttattctgccagcgtactgcaaagtggcgtaccttcccgcttctccgggtctgggagtggcactgattttaccctcacaattagcagcctgcaacccgaggacttcgctacatactactgccaacaaagtgtaatgatacccatgacattcgggcaaggcacaaaagtcgagataaagggaagtggaggaggtggctctatgccccgccgcgctgagaactgggatgaggccgaagttggtgctgaagaggccggagttgaagaatatgggccagaagaagatggcggtgaggaaagcggggctgaagagagcggtccagaggagtctggtccagaggaacttggagctgaggaggagatggaggccggacgtccacgtcctgtcctgcgatcagttaactcaagggagccctcacaggttatcttttgtaatcgaagccctcgcgtggttttgcccgtctggctcaacttcgatggtgaaccccaaccatacccaaccctcccccctggtaccgggcggaggattcattcctatcggggacacctttggctcttccgagacgctgggactcacgatggcctgttggtcaatcagaccgaactgtttgtgcccagcctgaacgtagacgggcagccaattttcgcaaacataacactgcccgtatatacattgaaagaaaggtgtcttcaggtggtacgcagtctggttaaaccagaaaactataggcgtctggatatcgtgcgcagcctctatgaggaccttgaagaccaccctaacgtgcaaaaggacctcgagcggctcactcaggagcgcatagctcatcagcgcatgggagatgaaaacctttactttcagggtgggagcggcggcagcggcgggagtcatcatcaccatcatcatcaccactga

SEQ ID NO: 19 - RNA, 1398 nt, synthetic construct
  source 1..1398: mol_type = other RNA
atggaagtgcaacttctcgaatctggaggggggttggtacaacccggcggcagcttgcgcttgtcctgtgctgccagtgggttcacattttctacattctctatgaactgggttagacaagcccctggcaaagggctggaatgggtgagctatataagtcgcacctccaaaactatttactatgcagatagtgtcaagggacgatttactatcagcagagataactctaagaacactctgtatctccagatgaattcccttcgagccgaagacaccgcagtatattactgtgctagagggcgcttcttcgactactgggggcaaggcactctggtaactgtcagtagcgggggttctgagggcaaaagttcaggatctgggtccgagtctaagtcaactggcgggagcgacatacaaatgactcagagccccagtagcctgagcgcctccgttggtgacagagtcactattacatgtcgggcatctcaatctatttcctcttatcttaactggtatcagcaaaagccaggcgaagcccccaaactcctgatatactccgctagtgttcttcagagtggcgttcctagtcgcttcagcggatccggaagtggcactgattttacacttacaattagttccttgcagcctgaagattttgccacatactactgtcagcaatcagtcatgattcccatgacctttgggcaagggaccaaagttgagatcaaaggctccggaggaggagggtctatggaaaacagatggcaagttatgatcgtttggcaagtagatcgtatgcgaatacgcacatggaaatcactggtaaagcaccacatgtatgtgtcaggcaaagcacgaggatggttttatcgtcatcactatgagtcaccacatccccgcatcagctctgaggtgcacataccactcggtgatgctcgtctggtcataactacctactggggcctccacactggtgaaagagattggcacctcggccaaggagtaagtatagaatggcgcaaaaagcgttattcaacccaagtggatcctgagttggcagatcagttgatccacttgtattactttgactgcttcagcgatagtgctattcggaaggccctcctcgggcacattgtaagcccacggtgcgagtatcaagctggtcataacaaggttggtagcctccagtacttggctttggctgcacttataacacccaaaaagataaaacctccactcccctcagtgactaaactcactgaggatcgttggaacaaaccccagaaaaccaaggggcacaggggttcacacaccatgaatggccacgagaatttgtatttccaagggggatccgggggcagtggagggtctcaccatcatcaccaccaccaccattga

SEQ ID NO: 20 - RNA, 19 nt, synthetic construct
  source 1..19: mol_type = other RNA
cagctaattcagaatcatt

SEQ ID NO: 21 - RNA, 19 nt, synthetic construct
  source 1..19: mol_type = other RNA
aatgattctgaattagctg